European Patent Application EP 4 260 686 A1, published October 18, 2023. Title: TOMATO LYCOPENE EPOXIDASE IMPROVING BETA-CAROTNE OR LUTEIN LEVEL AND USES THEREOF. Applicant: Kyungpook National University Industry-Academic Cooperation Foundation. The sequence listing filed with the application follows.

SEQUENCE LISTING (108 sequences)

SEQ ID NO: 1 - DNA, 1423 bp, M82
aaataattacaagtgttattaacattgaaaaagtccagataattaaaattagtacactacaacaatatgtttgtttgttcaatatttagtgtatagtaactacgatgatttgtttgtttgtcaaatttatagttgtatagtaattacaatgatatgtttgtttgccaaattatagggtaattgcaagtggactatttgattgtacaagtgtaattataaaattatatgaattttaaaaactaaaaagttatactagataaattaatcataaaaattaaaaatacaaagttttaatgaaaatcatgaaatatatgtttgacaaaaaaattaatattataaatatgttgtcataatattatagaaatatttgataaaaataatatattaagtctaactaaaaaaataaattacaatgtaaaatattgacgtaatattcctaaaacaaataaatttgaaaacataacataagttctaaattcgaaataaaaaatcaacatataatactctgatgttaaattcgacacaacatacacaaagatgattttaaaagaacaggaaaatgtatatccataatcttatgcaacaatgaattctattttaattttaaaaaatttaaaataataacaatgtttatatatatttgaaaaacgttagaataataataaaataaatgaaaaaaaaataaagagaagaaattaaaaagtaatccctatatgtcaaaaaatcacgaactcttaaaaattgaaaagtataattattcgtgtcaattatctagtgatccaaaataatataattatattaaattacaccaaatttaatcaacaaaatgatgtttattcgtaattttgtataaagaatgttacgataatttatagtctaaattcaaattatgataaagaagaattaaatatatacgtacataaacaaaaaaaagtttaaatcttgcaatctaggaataataatatctaatcattcgtatttaaattgagaaatgttaatacttctttcgttttaaaaaaaaatcttaatagtctatttaaaaaagaatgattactttttttttggtaatattttaattttttgaataatattttaattttaatttttcacatgacctatttaagaccacaaggttataagatatttttatacatttaatataattttaatttagatccacaaaattaaatattttctttattttcttaaactatatttaaaattaaactagataactctttttaaaaggaaagaaatattaacgaaataaataaaatgtgctaaataaatattcttgcatttggcccctcctgccaattgccagacttgaatattgtctctcgtgtttttttttattgtcatcctcgcaattttcacccaaaatcacacggtccaattggatccccaatttcggattgcgatg

SEQ ID NO: 2 - DNA, 1480 bp, LA317
aaataattacaagtgttattaacattgaaaaagtccagataattaaaattagtacactacaacaatatgtttgtttgttcaatatttagtgtatagtaactacgatgatttgtttgtttgtcaaatttatagttgtatagtaattacaatgatatgtttgtttgccaaattatagggtaattgcaagcgccaaccccgactcctccaccaaagaattctggtctggagctcattccgaagtggactatttgattgtacaagtgtaattataaaattatatgaattttaaaaattaaaaagttatactagataaattaatcataaaaattaaaaatacaaagttttaatgaaaatcatgaaatatatgtttgacaaaaaaattaatattataaatatgttgtcataatattatagaaatatttgataaaaataatatattaagtctaactaaaaaaataaattacaatgtaaaatatcgacgtaatattcctaaaacaaataaatttgaaaacataacataagttctaaattcgaaataaaaaatcaacatataatactctgatgttaaattcgacacaacatacacaaagatgattttaaaagaacaggaaaatgtatatccataatcttatgcaacaatgaattctattttaattttaaaaaatttaaaataataacaatgtttatatatatttgaaaaacgttagaataataataaaataaatgaaaaaaaataaagagaagaaattaaaaagtaatccctatatgtcaaaaaatcacgaactcctaaaaattgaaaagtataattattcgtgtcaattatctagtgatccaaaataatataattatattaaattacaccaaatttaatcaacaaaatgatgtttattcgtaattttgtataaagaatgttacgataatttatagtctaaattcaaattatgataaagaagaattaaatatatacgtacataaacaaaaagaagtttaaatcttgcaatctaggaataataatatctaatcattcgtatttaaattgagaaatgttaatacttctttcgttttaaaaaaaagatcttaatagtctatttaaaaaagaatgattactttttttggtaatattttaattttttgaataatattttaattttaatttttcacatgatctatttaagaccacaaggttataaaacaattttatacatttgatataattttaatttagatccacaaaattaaatattttctttattttcttaaactatatttaaaattaaactagataactctttttaaaaggaaagaaatattaacgaaataaataaaatgtgctaaataaatattcttgcatttggcccctcctgccaattgccagacttgaatattgtctctcgtgtttttttttttttttattgtcatcctcgcaattttcacccaaaatcacacggtccaattggatccccaatttcggatttcgatg

SEQ ID NO: 3 - DNA, 1480 bp, LA1412
aaataattacaagtgttattaacattgaaaaagtccagataattaaaattagtacactacaacaatatgtttgtttgttcaatatttagtgtatagtaactaagatgatttgtttgtttgtcaaatttatagttgtatagtaattacaatgatatgtttgtttgccaaattatagggtaattgcaagcgccaaccccgactcctccaccaaagaattctggtctggagctcattccgaagtggactatttgattgtacaagtgtaattataaaattatatgaattttaaaaattaaaaagttatactagataaattaatcataaaaattaaaaatacaaagttttaatgaaaatcatgaaatatatgtttgacaaaaaaattaatattataaatatgttgtcataatattatagaaatatttgataaaaataatatattaagtctaactaaaaaaataaattacaatgtaaaatatcgacgtaatattcctaaaacaaataaatttgaaaacataacataagttctaaattcgaaataaaaaatcaacatataatactctgatgttaaattcgacacaacatacacaaagatgattttaaaagaacaggaaaatgtatatccataatcttatgcaacaatgaattctattttaattttaaaaaatttaaaataataacaatgtttatatatatttgaaaaacgttagaataataataaaataaatgaaaaaaaataaagagaagaaattaaaaagtaatccctatatgtcaaaaaatcacgaactcctaaaaattgaaaagtataattattcgtgtcaattatctagtgatccaaaataatataattatattaaattacaccaaatttaatcaacaaaatgatgtttattcgtaattttgtataaagaatgttacgataatttatagtctaaattcaaattatgataaagaagaattaaatatatacgtacataaacaaaaagaagtttaaatcttgcaatctaggaataataatatctaatcattcgtatttaaattgagaaatgttaatacttctttcgttttaaaaaaaagatcttaatagtctatttaaaaaagaatgattactttttttggtaatattttaattttttgaataatattttaattttaatttttcacatgatctatttaagaccacaaggttataaaacaattttatacatttgatataattttaatttagatccacaaaattaaatattttctttattttcttaaactatatttaaaattaaactagataactctttttaaaaggaaagaaatattaacgaaataaataaaatgtgctaaataaatattcttgcatttggcccctcctgccaattgccagacttgaatattgtctctcgtgtttttttttttttttattgtcatcctcgcaattttcacccaaaatcacacggtccaattggatccccaatttcggatttcgatg

SEQ ID NO: 4 - DNA, 3217 bp, LA716
aaataattacaagtgttattaacattgaaaagtccagataattaaaattagtacactacaacaatatgtttgttaaatatttagtgaatagtaattacgatgatttatttgtttgttaaatttatagtgtatagtgattacaatgatatgtgttatattctaggtgttttgatgatcctcactaatgtggggacctggtccctggcagagtgctttcgtccagatacaaaggggtacagtcgtaaaagctgtcatgtcaggtgataggtgaaaagtgcagtatcatacaccaatagaaaagcggacgagattgtatgtttcagtatctcacaaatgcagggcttggtaccaggcagagtttcctccatcagatacataattggttacagctgtaaagttgtcacgtcagaggttggtaaggcgtcagtgtactacacaccaatcagaatggaggagggtgtttgtccaacggataataactctttatgtttgatacttttagcatgacaaacaccatattatattcattcatccaaagaaggaagtcagccagcaagccttttcaagaactcacaaagaagtttgcaagggacctggtccccgcaagactgcgaggtgaaaaggatgaaaagacagctgtcatctctgatgcgataggtgcacaacttttccaacagcaggccttcagccaatgggatggcttcaacgaatttgtgggaaattatattatctctttcaacaaacacaaattgaagacttggaaaattaaacttggattttctctgaaaattcacaagcttgaacagaaagccatcttcaaggaagaacattgctcaactcaacagaaggacctgatagagtaaagaagaatctttgttgtatttagagctttgtgtctatgtacttatattgtaaatttgttcctaatctataaaggattcagatatttgttttgggtttgtaaaagtctaaatcagttaaggttaactgatttagtgggcaacattgttttgttgcttagtcaaattctaagtaatctagagttaggtggtttagtgggcgatgtggtatccgcttagcaaattctaagttatctaggggtgatagcttagtgggcggcgttgtatccgcttaggctcttcaagtaataggtagattacttgatcgtgagattaataactttttctcacattgattgtaaccgggtttcacttttgcttgagaagattagtgaagacggttgtaaatcctgtgcagcaggtcatggttttactcccttgagcaaggaggtttccacgtaaattgcttgtgttgtgttcttcatattatttaatcttccgcactgttcttgctgtgtcaagggacctggtccgttgactggtagtggacgcacatattccaacaaatatgtttgtttgccaaattatagggtaattgcaagtgtactatttgattgcacaagtgtaattataaaattatatgaattttaaaaactaaaaagttatactagataaattaatcataaaaactaaaagtaccaaatttcaatgaacatcatgaaatgtatgtttgacaaaaagattaatattataaatatgatgtcataatattatagaaatatttgataaaaatagtatgttaagtctaactaaaaaaataaattacaatgtaaaatatcgacgtaatattcctaaaacaaatgaaattaaaaatataacataagttctaaatttaaaataaaaaatcaatatataatatactctgatgtcaaattcaacacaacatacacaaagataatttttttaaaagaaaaaaaaatgtatgtgcataatcttattcaacaatgaattctattttaattttaaaaaattaaaataatgacaatgtgtatatatatttgaaaaacattagaataataaaaataaataataaaataaaatggaaaaaaaataaagagaagaaattagaaagtaatccctgtatgtcaaaaagtcacaaactcctgaagagtgtaattattcgtgtcaattacctaataatctaaaataaatatgtcagacaatataattatactaaattacaccaaatttaattaacaaaataatgtttatttgtaattttgtactaagaatgttacaataatttatagtctaaattcaaattatgataaagaagcattaaatatatacgtacataaacaaaaagtagtttaaatcttacgatctagaaataatatctaatcattcgtatttaaattgagaaatgttaatactttttttcgtttaaaaaattgattttattttttttagtttattttaaaaagaatgattacttttcttttttgacaatattttaatttctttttttggtaatatttaaattttaattttccacgtgatatgtttaagataaaaaaattataagatattttggtacatatgaagctagcgtttgactataaattttcaaatattcttggcaaatattatttgagtgaaaatttggttgggaaatatatttcacctttttagaaaaatataatttataaccataagttttaaaaactattaaaactaactataagtttatacaataacaaatagtttccatcacactagagcaatgtggtaatttggagcgagtgcaacaagtatcattccatacatcgtgaagtagacgaagcacatgattttattaccttgagttaatttttcatcattttcatcaacaatcatatcattatttaatattcactaaatatttcatcactattttggtgttcacgtaaaaaaattatgtaatacaacacaaacaactactaaaagggtgtttttgtaaaagataaaagtttgggataaaattttaatattcaaaagatcccaaataatgagatttggcccaaatactagaaaaaattagtatttgggaatttgggatatttgccaaaaatgtttgccaaataatgacaaattgtatggacaaacattaaatatttttttcttaaattctgtttgaaattaaattagatcattctttttaaaacgaaaaaatattaactaaagaaataaaatgtgctaaataaatattcttgcatttggcccctcctgccaattgccagacttgaatattgtctctcgtgttgtttttttttgtcatcctcgcaattttcacccaaaatcaaacggtccaattggatcccaaatttcgtatttcgatg

SEQ ID NO: 5 - DNA, 24 bp, Artificial Sequence
  T1117-F
caaggctgaaaccaaaagacattg

SEQ ID NO: 6 - DNA, 24 bp, Artificial Sequence
  T1117-R
acatttaaatgctttgtcgtctgc

SEQ ID NO: 7 - DNA, 24 bp, Artificial Sequence
  97-F
cctgttaactacttcttgactatg

SEQ ID NO: 8 - DNA, 23 bp, Artificial Sequence
  97-R
tcagtgtttcacaatctaagtgc

SEQ ID NO: 9 - DNA, 23 bp, Artificial Sequence
  98-F
tacagccttccatctatgcaaag

SEQ ID NO: 10 - DNA, 21 bp, Artificial Sequence
  98-R
cctatttgttagacggcgagg

SEQ ID NO: 11 - DNA, 24 bp, Artificial Sequence
  At1g60640-F
tctgacagggggaaatgaatcttc

SEQ ID NO: 12 - DNA, 29 bp, Artificial Sequence
  At1g60640-R
acttcattgaaagagctatcttcactctc

SEQ ID NO: 13 - DNA, 24 bp, Artificial Sequence
  01-F
tgtgtgcttattgccacttatata

SEQ ID NO: 14 - DNA, 24 bp, Artificial Sequence
  01-R
tgttcttgaggaaaacaatagagc

SEQ ID NO: 15 - DNA, 24 bp, Artificial Sequence
  02-F
tccaattcacgttaggtaattaag

SEQ ID NO: 16 - DNA, 23 bp, Artificial Sequence
  02-R
ctgtacctcctcattatatttgg

SEQ ID NO: 17 - DNA, 23 bp, Artificial Sequence
  04-F
ggctcaggatcaagttcaatatg

SEQ ID NO: 18 - DNA, 22 bp, Artificial Sequence
  04-R
cttcacatcactctcaggcaac

SEQ ID NO: 19 - DNA, 24 bp, Artificial Sequence
  09-F
atagatcaatttagtgcagtagtg

SEQ ID NO: 20 - DNA, 24 bp, Artificial Sequence
  09-R
agtaattttgagtaatggaggaag

SEQ ID NO: 21 - DNA, 23 bp, Artificial Sequence
  10-F
gtgaatgtgtaagagagttgtcc

SEQ ID NO: 22 - DNA, 23 bp, Artificial Sequence
  10-R
actattgtgttgtgccgaaatcc

SEQ ID NO: 23 - DNA, 23 bp, Artificial Sequence
  13-F
gaattattctgcttctaaggctc

SEQ ID NO: 24 - DNA, 23 bp, Artificial Sequence
  13-R
atgtctttcgagtactagtcatg

SEQ ID NO: 25 - DNA, 25 bp, Artificial Sequence
  RnaB-F
gaatatgatttatcaacaagtatcc

SEQ ID NO: 26 - DNA, 22 bp, Artificial Sequence
  RnaB-R
gcatgattggtgttagcgggac

SEQ ID NO: 27 - DNA, 22 bp, Artificial Sequence
  TG276-F
ctggtgctgctcttgctcatac

SEQ ID NO: 28 - DNA, 22 bp, Artificial Sequence
  TG276-R
aatccctttcgatgacgtgaac

SEQ ID NO: 29 - DNA, 23 bp, Artificial Sequence
  RnaP-F
gttcatccgcaacctattgtacc

SEQ ID NO: 30 - DNA, 23 bp, Artificial Sequence
  RnaP-R
tgcactctcattagctacatcac

SEQ ID NO: 31 - DNA, 24 bp, Artificial Sequence
  U582871-F
taacagaattaattcgtgtgattg

SEQ ID NO: 32 - DNA, 22 bp, Artificial Sequence
  U582871-R
agcaagaaacgtgtctgttcag

SEQ ID NO: 33 - DNA, 23 bp, Artificial Sequence
  26D15-3-F
aaagagttgccttctttaacatg

SEQ ID NO: 34 - DNA, 22 bp, Artificial Sequence
  26D15-3-R
ggtttgtatatccctcctcatc

SEQ ID NO: 35 - DNA, 23 bp, Artificial Sequence
  2B-F
cgtggactacctaactagcagac

SEQ ID NO: 36 - DNA, 22 bp, Artificial Sequence
  2B-R
tgtgtgttggacgtaggccatg

SEQ ID NO: 37 - DNA, 23 bp, Artificial Sequence
  T0888-F
gaatcggagcaagtaactcagtc

SEQ ID NO: 38 - DNA, 24 bp, Artificial Sequence
  T0888-R
gagtttgaggttactcgttatgtc

SEQ ID NO: 39 - DNA, 23 bp, Artificial Sequence
  T1238-F
gaattcttgcaagctacatgagg

SEQ ID NO: 40 - DNA, 24 bp, Artificial Sequence
  T1238-R
acaagatgtcctttcttaatagtg

SEQ ID NO: 41 - DNA, 23 bp, Artificial Sequence
  U562933-F
gcacacatggttacctgattacc

SEQ ID NO: 42 - DNA, 23 bp, Artificial Sequence
  U562933-R
ctgagtgaccaaatgtgtgtacc

SEQ ID NO: 43 - DNA, 22 bp, Artificial Sequence
  46485-3-F
gggagataactcgagggctcag

SEQ ID NO: 44 - DNA, 27 bp, Artificial Sequence
  46485-3-R
cgccaactttatacccaatgaatgtgc

SEQ ID NO: 45 - DNA, 22 bp, Artificial Sequence
  U572717-F
atccatccgattatcccttccg

SEQ ID NO: 46 - DNA, 22 bp, Artificial Sequence
  U572717-R
tgagactgaactcgccatgctc

SEQ ID NO: 47 - DNA, 23 bp, Artificial Sequence
  U572498-F
gatcaattcgtgtcaattacagg

SEQ ID NO: 48 - DNA, 23 bp, Artificial Sequence
  U572498-R
gtgatcaagttggctgtgtgaag

SEQ ID NO: 49 - DNA, 25 bp, Artificial Sequence
  2A-F
cttcatgattacactttgccattat

SEQ ID NO: 50 - DNA, 23 bp, Artificial Sequence
  2A-R
gattacctcaggagggcttaacc

SEQ ID NO: 51 - DNA, 21 bp, Artificial Sequence
  U569822-F
aacggagaaagtgggatcagc

SEQ ID NO: 52 - DNA, 22 bp, Artificial Sequence
  U569822-R
ttggcgctttgtgagcctgtag

SEQ ID NO: 53 - DNA, 22 bp, Artificial Sequence
  CT196-F
acaacagctgctattactaccg

SEQ ID NO: 54 - DNA, 22 bp, Artificial Sequence
  CT196-R
ttcttgccggagatagaggtgg

SEQ ID NO: 55 - DNA, 22 bp, Artificial Sequence
  T0869-F
gttacgctagggcatttccgtc

SEQ ID NO: 56 - DNA, 23 bp, Artificial Sequence
  T0869-R
gataccaatcgaagtaacagcag

SEQ ID NO: 57 - DNA, 20 bp, Artificial Sequence
  SSR40-F
tgcaggtatgtctcacacca

SEQ ID NO: 58 - DNA, 20 bp, Artificial Sequence
  SSR40-R
tgcaacaactggataggtcg

SEQ ID NO: 59 - DNA, 50 bp, Artificial Sequence
  bc2.1-attB1
ggggacaagtttgtacaaaaaagcaggcttgaagacggagtcagattaag

SEQ ID NO: 60 - DNA, 50 bp, Artificial Sequence
  bc2.1-attB2
ggggaccactttgtacaagaaagctgggtgagtctgactagatttaaatg

SEQ ID NO: 61 - DNA, 22 bp, Artificial Sequence
  bc2.1-mTrcHis2-F
ttcatgatggataagtatattg

SEQ ID NO: 62 - DNA, 21 bp, Artificial Sequence
  bc2.1-mTrcHis2-R
ttaatctgactccgtcttcac

SEQ ID NO: 63 - DNA, 22 bp, Artificial Sequence
  qRT-F
ctgctcttgctcatacccttgc

SEQ ID NO: 64 - DNA, 23 bp, Artificial Sequence
  qRT-R
ggattgttggcgaattgcttcag

SEQ ID NO: 65 - DNA, 27 bp, Artificial Sequence
  cis1-F
aaataattacaagtgttattaacattg

SEQ ID NO: 66 - DNA, 24 bp, Artificial Sequence
  cis1-R
tgtttgtatttataagaagcatcg

SEQ ID NO: 67 - DNA, 23 bp, Artificial Sequence
  cDNA1-F
ttgtcatcctcgcaattttcacc

SEQ ID NO: 68 - DNA, 23 bp, Artificial Sequence
  cDNA1-R
cttaatctgactccgtcttcacg

SEQ ID NO: 69 - DNA, 32 bp, Artificial Sequence
  CYC-B-AscI-F
ggcgcgccatggaaactcttctcaagcctttt

SEQ ID NO: 70 - DNA, 32 bp, Artificial Sequence
  CYC-B-AscI-R
ggcgcgccaaggctctctattgctagattgcc

SEQ ID NO: 71 - DNA, 32 bp, Artificial Sequence
  bc2.1-AscI-F
ggcgcgccatgcttcttataaatacaaacaat

SEQ ID NO: 72 - DNA, 32 bp, Artificial Sequence
  bc2.1-AscI-R
ggcgcgccatctgactccgtcttcacgggagg

SEQ ID NO: 73 - DNA, 35 bp, Artificial Sequence
  bc2.1-GFP-F
ggcgcgcctctagaatgcttcttataaatacaaac

SEQ ID NO: 74 - DNA, 34 bp, Artificial Sequence
  bc2.1-GFP-R
ggcgcgccgtcgacatctgactccgtcttcacgg

SEQ ID NO: 75 - DNA, 25 bp, Artificial Sequence
  35S-F
cccaagaaggttaaagatgcagtca

SEQ ID NO: 76 - DNA, 25 bp, Artificial Sequence
  35S-R
gctttgaagacgtggttggaacgtc

SEQ ID NO: 77 - DNA, 20 bp, Artificial Sequence
  PSY1-F
tggcccaaacgcatcatata

SEQ ID NO: 78 - DNA, 21 bp, Artificial Sequence
  PSY1-R
caccatcgagcatgtcaaatg

SEQ ID NO: 79 - DNA, 21 bp, Artificial Sequence
  PSY2-F
gttgatggccctaatgcatca

SEQ ID NO: 80 - DNA, 20 bp, Artificial Sequence
  PSY2-R
tcaagcatatcaaatggccg

SEQ ID NO: 81 - DNA, 25 bp, Artificial Sequence
  PDS-F
gtgcattttgatcatcgcattgaac

SEQ ID NO: 82 - DNA, 21 bp, Artificial Sequence
  PDS-R
gcaaagtctctcaggattacc

SEQ ID NO: 83 - DNA, 19 bp, Artificial Sequence
  ZDS-F
ttggagcgttcgaggcaat

SEQ ID NO: 84 - DNA, 24 bp, Artificial Sequence
  ZDS-R
agaaatctgcatctggcgtataga

SEQ ID NO: 85 - DNA, 21 bp, Artificial Sequence
  Z-ISO-F
tatgaggattaccaggcatcc

SEQ ID NO: 86 - DNA, 20 bp, Artificial Sequence
  Z-ISO-R
acagcgtgtgagctaagcac

SEQ ID NO: 87 - DNA, 20 bp, Artificial Sequence
  CRTISO-F
ttttggcggaatcaactacc

SEQ ID NO: 88 - DNA, 20 bp, Artificial Sequence
  CRTISO-R
gaaagcttcactcccacagc

SEQ ID NO: 89 - DNA, 27 bp, Artificial Sequence
  CYC-B-F
tgttattgaggaagagaaatgtgtgat

SEQ ID NO: 90 - DNA, 24 bp, Artificial Sequence
  CYC-B-R
tcccaccaatagccataacatttt

SEQ ID NO: 91 - DNA, 21 bp, Artificial Sequence
  LCY-B-F
tcgttggaatcggtggtacag

SEQ ID NO: 92 - DNA, 21 bp, Artificial Sequence
  LCY-B-R
agctagtgtccttgccaccat

SEQ ID NO: 93 - DNA, 23 bp, Artificial Sequence
  CCD1A-F
tggattatgacaaacgattgacg

SEQ ID NO: 94 - DNA, 24 bp, Artificial Sequence
  CCD1A-R
ttggatataaccctataagtgatg

SEQ ID NO: 95 - DNA, 23 bp, Artificial Sequence
  CCD1B-F
ggattacgataaaaggttgcaac

SEQ ID NO: 96 - DNA, 24 bp, Artificial Sequence
  CCD1B-R
cttggatatgactctatatgtagc

SEQ ID NO: 97 - DNA, 21 bp, Artificial Sequence
  CRTR-b1-F
agatgggcacacaaagcactg

SEQ ID NO: 98 - DNA, 20 bp, Artificial Sequence
  CRTR-b1-R
gcgaaaacgtcgttcagctc

SEQ ID NO: 99 - DNA, 20 bp, Artificial Sequence
  CRTR-b2-F
tttcagcctccgctagttcc

SEQ ID NO: 100 - DNA, 21 bp, Artificial Sequence
  CRTR-b2-R
cggagagaagaacagaaccgg

SEQ ID NO: 101 - DNA, 23 bp, Artificial Sequence
  ZEP-F
ttgatggtatttctggcaactgg

SEQ ID NO: 102 - DNA, 22 bp, Artificial Sequence
  ZEP-R
accaacagcacgtgcaaggatc

SEQ ID NO: 103 - DNA, 23 bp, Artificial Sequence
  VDE-F
tgcctgaaacgattatacctgag

SEQ ID NO: 104 - DNA, 22 bp, Artificial Sequence
  VDE-R
ccgctctccttcttccactttc

SEQ ID NO: 105 - DNA, 23 bp, Artificial Sequence
  NCED1-F
gggatggtttagaatatacgtcc

SEQ ID NO: 106 - DNA, 23 bp, Artificial Sequence
  NCED1-R
ggttctctgagaatctctcacac

SEQ ID NO: 107 - DNA, 19 bp, Artificial Sequence
  18S-F
cggagagggagcctgagaa

SEQ ID NO: 108 - DNA, 23 bp, Artificial Sequence
  18S-R
cccgtgttaggattgggtaattt